European Patent Specification EP 3 896 172 B1, published August 9, 2023. Title: Method for Detecting Genomic Rearrangements. Applicant: Inivata Limited. Application PCT/GB2018/051688. The sequence listing filed with the application follows.

SEQUENCE LISTING (8 sequences)

SEQ ID NO: 1 - DNA, 34 bp, Artificial Sequence
  EML4-ALK gene fusion
gaagttcctatactttctagagaataggaacttc

SEQ ID NO: 2 - DNA, 108 bp, Artificial Sequence
  Primer Set 1
ttaattaaatgtttttcaaatccattcacctgaatgtctaagcttggcaggaagttcctatactttctagagaataggaacttcggaataggaacttcatatggtgcc

SEQ ID NO: 3 - DNA, 68 bp, Artificial Sequence
  Primer Set 2
aggaagttcctatactttctagagaataggaacttcggaataggaacttcatatggtgccatccctca

SEQ ID NO: 4 - DNA, 499 bp, Artificial Sequence
  ROS1-CD74 gBlock Sequence
cgccaaggtcacagctgctgccaagagagccttgggcgtttcccacctcatggacaatgcagactaggatgtttttagacccaaagacagagtgctgtttctatcccggtgctgtctctaatttgctatgtaactttggacaagtccccttccctctaggattcagggtcctgaagtagaaggtcaaagggccaccctgcctggggcctcagtttctgcatcagattcatagaaggcaccttacatgctattgtcatgtatattttctgtatttattattttttgcagaaagagcacttcaaataatttacagaaccagaatttaaggtggagatgacatttaatggatcctgcagtagtgtttgcacatggaagtccaaaaacctgaaaggaatatttcagttcagagtagtagctgcaaataatctagggtttggtgaatatagtggaatcagtgagaatattatattagttggaggtatgttaccatgtctgtcta

SEQ ID NO: 5 - DNA, 104 bp, Artificial Sequence
  CD74_E6-I6_10 (fw) ROS1_I32_E33_414 (rv) sequence read
ttacatgctattgtcatgtatattttctgtatttattattttttgcagaaagagcacttcaaataatttacagaaccagaatttaaggtggaagatgacattta

SEQ ID NO: 6 - DNA, 110 bp, Artificial Sequence
  CD74_E6-I6_9 (fw) ROS1_I32_E33_414 (rv) sequence read
ccctgcctggggcctcagtttctgcatcagattcatagaaggcaccttacatgctattgtcatgtatattttctgtatttattattttttgcagaaagagcacttcaaat

SEQ ID NO: 7 - DNA, 499 bp, Artificial Sequence; identical to SEQ ID NO: 4
  CD74_E6-I6_10/ROS1_I32_E33_414 Read

SEQ ID NO: 8 - DNA, 499 bp, Artificial Sequence; identical to SEQ ID NO: 4
  CD74_E6-I6_9/ROS1_I32_E33_414 Read